European Patent Application EP 4 609 880 A1, published September 3, 2025. Title: PREPARATION CONTAINING ANTI-NECTIN-4 ANTIBODY-DRUG CONJUGATE AND USE THEREOF. Applicant: JIANGSU MABWELL HEALTH PHARMACEUTICAL R&D CO., LTD. The sequence listing filed with the application follows.

SEQUENCE LISTING (10 sequences)

SEQ ID NO: 1 - protein, 449 aa, synthetic construct
EVQLQESGPGLVKPSETLSLTCTVSGFSLIDYGVSWIRQPPGKGLEWIGVIWGGGKIYYNSVLKSRVTISKDNSKSQVSLKLSSVTAADTAVYYCAKQGGLLFYAMDYWGQGTLVTVSSASTKGPSVFPLAPSSKSTSGGTAALGCLVKDYFPEPVTVSWNSGALTSGVHTFPAVLQSSGLYSLSSVVTVPSSSLGTQTYICNVNHKPSNTKVDKRVEPKSCDKTHTCPPCPAPELLGGPSVFLFPPKPKDTLMISRTPEVTCVVVDVSHEDPEVKFNWYVDGVEVHNAKTKPREEQYNSTYRVVSVLTVLHQDWLNGKEYKCKVSNKALPAPIEKTISKAKGQPREPQVYTLPPSREEMTKNQVSLTCLVKGFYPSDIAVEWESNGQPENNYKTTPPVLDSDGSFFLYSKLTVDKSRWQQGNVFSCSVMHEALHNHYTQKSLSLSPGK

SEQ ID NO: 2 - protein, 119 aa, synthetic construct
EVQLQESGPGLVKPSETLSLTCTVSGFSLIDYGVSWIRQPPGKGLEWIGVIWGGGKIYYNSVLKSRVTISKDNSKSQVSLKLSSVTAADTAVYYCAKQGGLLFYAMDYWGQGTLVTVSS

SEQ ID NO: 3 - protein, 5 aa, synthetic construct
DYGVS

SEQ ID NO: 4 - protein, 16 aa, synthetic construct
VIWGGGKIYYNSVLKS

SEQ ID NO: 5 - protein, 11 aa, synthetic construct
QGGLLFYAMDY

SEQ ID NO: 6 - protein, 220 aa, synthetic construct
DIVMTQSPDSLAVSLGERATINCKSSQSLLNTYSQKNYLAWYQQKPGQPPKLLIYFASTRESGVPDRFSGSGSGTDFTLTISSLQAEDVAVYYCQQHYNTPFTFGGGTKVEIKRTVAAPSVFIFPPSDEQLKSGTASVVCLLNNFYPREAKVQWKVDNALQSGNSQESVTEQDSKDSTYSLSSTLTLSKADYEKHKVYACEVTHQGLSSPVTKSFNRGEC

SEQ ID NO: 7 - protein, 113 aa, synthetic construct
DIVMTQSPDSLAVSLGERATINCKSSQSLLNTYSQKNYLAWYQQKPGQPPKLLIYFASTRESGVPDRFSGSGSGTDFTLTISSLQAEDVAVYYCQQHYNTPFTFGGGTKVEIK

SEQ ID NO: 8 - protein, 17 aa, synthetic construct
KSSQSLLNTYSQKNYLA

SEQ ID NO: 9 - protein, 7 aa, synthetic construct
FASTRES

SEQ ID NO: 10 - protein, 9 aa, synthetic construct
QQHYNTPFT